European Patent Specification EP 3 624 593 B1, published November 12, 2025. Title: BETA-GALACTOSIDASE COMPOSITIONS. Applicant: Novozymes A/S Tams, Jeppe Wegener. The sequence listing filed with the application follows.

SEQUENCE LISTING (15 sequences)

SEQ ID NO: 1 - protein, 1304 aa, Artificial sequence
  Synthetic construct
VEDATRSDSTTQMSSTPEVVYSSAVDSKQNRTSDFDANWKFMLSDSVQAQDPAFDDSAWQQVDLPHDYSITQKYSQSNEAESAYLPGGTGWYRKSFTIDRDLAGKRIAINFDGVYMNATVWFNGVKLGTHPYGYSPFSFDLTGNAKFGGENTIVVKVENRLPSSRWYSGSGIYRDVTLTVTDGVHVGNNGVAIKTPSLATQNGGNVTMNLTTKVANDTKAAANITLKQTVFPKGGKTDAAIGTVTTASKSIAAGASADVTSTITAASPKLWSIKNPNLYTVRTEVLNGGKVLDTYDTEYGFRWTGFDATSGFSLNGEKVKLKGVSMHHDQGSLGAVANRRAIERQVEILQKMGVNSIRTTHNPAAKALIDVCNEKGVLVVEEVFDMWNRSKNGNTEDYGKWFGQAIAGDNAVLGGDKDETWAKFDLTSTINRDRNAPSVIMWSLGNEMMEGISGSVSGFPATSAKLVAWTKAADSTRPMTYGDNKIKANWNESNTMGDNLTANGGVVGTNYSDGANYDKIRTTHPSWAIYGSETASAINSRGIYNRTTGGAQSSDKQLTSYDNSAVGWGAVASSAWYDVVQRDFVAGTYVWTGFDYLGEPTPWNGTGSGAVGSWPSPKNSYFGIVDTAGFPKDTYYFYQSQWNDDVHTLHILPAWNENVVAKGSGNNVPVVVYTDAAKVKLYFTPKGSTEKRLIGEKSFTKKTTAAGYTYQVYEGADKDSTAHKNMYLTWNVPWAEGTISAEAYDENNRLIPEGSTEGNASVTTTGKAAKLKADADRKTITADGKDLSYIEVDVTDANGHIVPDAANRVTFDVKGAGKLVGVDNGSSPDHDSYQADNRKAFSGKVLAIVQSTKEAGEITVTAKADGLQSSTVKIATTAVPGTSTEKTVRSFYYSRNYYVKTGNKPILPSDVEVRYSDGTSDRQNVTWDAVSDDQIAKAGSFSVAGTVAGQKISVRVTMIDEIGALLNYSASTPVGTPAVLPGSRPAVLPDGTVTSANFAVDWTKPADTVYNTAGTVKVPGTATVFGKEFKVTATIRVQRSQVTIGSSVSGNALRLTQNIPADKQSDTLDAIKDGSTTVDANTGGGANPSAWTNWAYSKAGHNTAEITFEYATEQQLGQIVMYFFRDSNAVRFPDAGKTKIQISADGKNWTDLAATETIAAQESSERVKPYTYDFAPVGATFVKVTVTNADTTTPSGVVCAGLTEIELKTATSKFVTNTSAALSSLTVNGTKVSDSVLAAGSYNTPAIIADVKAEGEGNASVTVLPAHDNVIRVITESEDHVTRKTFTINLGTEQEFPADSDERD

SEQ ID NO: 2 - protein, 1931 aa, Artificial sequence
  Synthetic construct
MKKPLGKIVASTALLISVAFSSSIASAAVEDATRSDSTTQMSSTPEVAYSSAVDSKQNRTSDFDANWKFMLSDSVQAQDPAFDDSAWQQVDLPHDYSITQKYSQSNEAESAYLPGGTGWYRKSFTIDRDLAGKRIAINFDGVYMNATVWFNGVKLGTHPYGYSPFSFDLTGNAKFGGENTIVVKVENRLPSSRWYSGSGIYRDVTLTVTDGVHVGNNGVAIKTPSLATQNGGDVTMNLTTKVANDTEAAANITLKQTVFPKGGKTDAAIGTVTTASKSIAAGASADVTSTITAASPKLWSIKNPNLYTVRTEVLNGGKVLDTYDTEYGFRWTGFDATSGFSLNGEKVKLKGVSMHHDQGSLGAVANRRAIERQVEILQKMGVNSIRTTHNPAAKALIDVCNEKGVLVVEEVFDMWNRSKNGNTEDYGKWFGQAIAGDNAVLGGDKDETWAKFDLTSTINRDRNAPSVIMWSLGNEMMEGISGSVSGFPATSAKLVAWTKAADSTRPMTYGDNKIKANWNESNTMGDNLTANGGVVGTNYSDGANYDKIRTTHPSWAIYGSETASAINSRGIYNRTTGGAQSSDKQLTSYDNSAVGWGAVASSAWYDVVQRDFVAGTYVWTGFDYLGEPTPWNGTGSGAVGSWPSPKNSYFGIVDTAGFPKDTYYFYQSQWNDDVHTLHILPAWNENVVAKGSGNNVPVVVYTDAAKVKLYFTPKGSTEKRLIGEKSFTKKTTAAGYTYQVYEGSDKDSTAHKNMYLTWNVPWAEGTISAEAYDENNRLIPEGSTEGNASVTTTGKAAKLKADADRKTITADGKDLSYIEVDVTDANGHIVPDAANRVTFDVKGAGKLVGVDNGSSPDHDSYQADNRKAFSGKVLAIVQSTKEAGEITVTAKADGLQSSTVKIATTAVPGTSTEKTVRSFYYSRNYYVKTGNKPILPSDVEVRYSDGTSDRQNVTWDAVSDDQIAKAGSFSVAGTVAGQKISVRVTMIDEIGALLNYSASTPVGTPAVLPGSRPAVLPDGTVTSANFAVHWTKPADTVYNTAGTVKVPGTATVFGKEFKVTATIRVQRSQVTIGSSVSGNALRLTQNIPADKQSDTLDAIKDGSTTVDANTGGGANPSAWTNWAYSKAGHNTAEITFEYATEQQLGQIVMYFFRDSNAVRFPDAGKTKIQISADGKNWTDLAATETIAAQESSDRVKPYTYDFAPVGATFVKVTVTNADTTTPSGVVCAGLTEIELKTATSKFVTNTSAALSSLTVNGTKVSDSVLAAGSYNTPAIIADVKAEGEGNASVTVLPAHDNVIRVITESEDHVTRKTFTINLGTEQEFPADSDERDYPAADMTVTVGSEQTSGTATEGPKKFAVDGNTSTYWHSNWTPTTVNDLWIAFELQKPTKLDALRYLPRPAGSKNGSVTEYKVQVSDDGTNWTDAGSGTWTTDYGWKLAEFNQPVTTKHVRLKAVHTYADSGNDKFMSASEIRLRKAVDTTDISGATVTVPAKLTVDRVDADHPATFATKDVTVTLGDATLRYGVDYLLDYAGNTAVGKATVTVRGIDKYSGTVAKTFTIELKNAPAPEPTLTSVSVKTKPSKLTYVVGDAFDPAGLVLQLNYDDDSTGTVTWNTQTAGDFTFKPALDAKLKVTDKTVTVTYQGKSAVIDITVSQPAPTVSKTDLDKAIKAIEAKNPDSSKYTADSWKTFADAMAHAKAVIADDSATQQDVDNALKALTDAYAGLTEKTPEPAPVSKSELDKKIKAIEAEKLDGSKYTAESWKAFETALAHAKAVIASDSATQQNVDAALGALTSARDGLTEKGEVKPDPKPEPGTVDKAALDKAVKKVEAEKLDGSKYTADSWKAFETALAHAKAVIGNANSTQFDIDNALSMLNDARAALKEKPGRIIAIIDGSALSKTGASVAIIASVAAAMLAVGAGVMALRRKRS

SEQ ID NO: 3 - protein, 1341 aa, Artificial sequence
  Synthetic construct
MKKPLGKIVASTALLISVAFSSSIASAIEDATRSDSTTQMSSTPEVAYSSAVDSKQNRTSDFDANWKFMLSDSVQAQDPAFDDSAWQQVDLPHDYSITQKYSQSNEAESAYLPGGTGWYRKSFTIDRDLAGKRIAINFDGVYMNATVWFNGVKLGTHPYGYSPFSFDLTGNAKFGGENTIVVKVENRLPSSRWYSGSGIYRDVTLTVTDGVHVGNNGVAIKTPSLATQNGGDVTMNLTTKVANDTEAAANITLKQTVFPKGGKTDAAIGTVTTASKSIAAGASADVTSTITAASPKLWSIKNPNLYTVRTEVLNGGKVLDTYDTEYGFRWTGFDATSGFSLNGEKVKLKGVSMHHDQGSLGAVANRRAIERQVEILQKMGVNSIRTTHNPAAKALIDVCNEKGVLVVEEVFDMWNRSKNGNTEDYGKWFGQAIAGDNAVLGGDKDETWAKFDLTSTINRDRNAPSVIMWSLGNEMMEGISGSVSGFSATSAKLVAWTKAADSTRPMTYGDNKIKANWNESNTMGDNLTANGGVVGTNYSDGANYDKIRTTHPSWAIYGSETASAINSRGIYNRTTGGAQSSDKQLTSYDNSAVGWGAVASSAWYDVVQRDFVAGTYVWTGFDYLGEPTPWNGTGSGAVGSWPSPKNSYFGIVDTAGFPKDTYYFYQSQWNDDVHTLHILPAWNENVVAKGSGNNVPVVVYTDAAKVKLYFTPKGSTEQRLIGEKSFTKKTTAAGYTYQVYEGSDKDSTAHKNMYLTWNVPWAEGTISAEAYDENNRLIPEGSTEGNASVTTTGKAAKLKADADRKTITADGKDLSYIEVDVTDANGHIVPDAANRVTFDVKGAGKLVGVDNGSSPDHDSYQADNRKAFSGKVLAIVQSTKEAGEITVTAKADGLQSSTVKIATTAVPGTSTEKTVRSFYYSRNYYVKTGNKPILPSDVEVRYSDGTSDRQNVTWDAVSDDQIAKAGSFSVAGTVAGQKISVRVTMIDEIGALLNYSASTPVGTPAVLPGSRPAVLPDGTVTSANFAVHWTKPADTVYNTAGTVKVPGTATVFGKEFKVTATIRVQRSQVTIGSSVSGNALRLTQNIPADKQSDTLDAIKDGSTTVDANTGGGANPSAWTNWAYSKAGHNTAEITFEYATEQQLGQIVMYFFRDSNAVRFPDAGKTKIQISADGKNWTDLAATETIAAQESSDRVKPYTYDFAPVGATFVRVTVTNADTTTPSGVVCAGLTEIELKTATSKFVANTSAALSSLTVNGTKVSDSVLAAGSYNTPAIIADVKAEGEGNASVTVLPAHDNVIRVITESEDHVTRKTFTINLGTEQEFPADSDERDQHQHQHQHQQ

SEQ ID NO: 4 - protein, 1752 aa, Artificial sequence
  Synthetic construct
MAVRRLGGRIVAFAATVALSIPLGLLTNSAWAVEDATRSDSTTQMSSTPEVVYSSAVDSKQNRTSDFDANWKFMLSDSVQAQDPAFDDSAWQQVDLPHDYSITQKYSQSNEAESAYLPGGTGWYRKSFTIDRDLAGKRIAINFDGVYMNATVWFNGVKLGTHPYGYSPFSFDLTGNAKFGGENTIVVKVENRLPSSRWYSGSGIYRDVTLTVTDGVHVGNNGVAIKTPSLATQNGGDVTMNLTTKVANDTEAAANITLKQTVFPKGGKTDAAIGTVTTASKSIAAGASADVTSTITAASPKLWSIKNPNLYTVRTEVLNGGKVLDTYDTEYGFRWTGFDATSGFSLNGEKVKLKGVSMHHDQGSLGAVANRRAIERQVEILQKMGVNSIRTTHNPAAKALIDVCNEKGVLVVEEVFDMWNRSKNGNTEDYGKWFGQAIAGDNAVLGGDKDETWAKFDLTSTINRDRNAPSVIMWSLGNEMMEGISGSVSGFPATSAKLVAWTKAADSTRPMTYGDNKIKANWNESNTMGDNLTANGGVVGTNYSDGANYDKIRTTHPSWAIYGSETASAINSRGIYNRTTGGAQSSDKQLTSYDNSAVGWGAVASSAWYDVVQRDFVAGTYVWTGFDYLGEPTPWNGTGSGAVGSWPSPKNSYFGIVDTAGFPKDTYYFYQSQWNDDVHTLHILPAWNENVVAKGSGNNVPVVVYTDAAKVKLYFTPKGSTEKRLIGEKSFTKKTTAAGYTYQVYEGSDKDSTAHKNMYLTWNVPWAEGTISAEAYDENNRLIPEGSTEGNASVTTTGKAAKLKADADRKTITADGKDLSYIEVDVTDANGHIVPDAANRVTFDVKGAGKLVGVDNGSSPDHDSYQADNRKAFSGKVLAIVQSTKEAGEITVTAKADGLQSSTVKIATTAVPGTSTEKTVRSFYYSRNYYVKTGNKPILPSDVEVRYSDGTSDRQNVTWDAVSDDQIAKAGSFSVAGTVAGQKISVRVTMIDEIGALLNYSASTPVGTPAVLPGSRPAVLPDGTVTSANFAVHWTKPADTVYNTAGTVKVPGTATVFGKEFKVTATIRVQRSQVTIGSSVSGNALRLTQNIPADKQSDTLDAIKDGSTTVDANTGGGANPSAWTNWAYSKAGHNTAEITFEYATEQQLGQIVMYFFRDSNAVRFPDAGKTKIQISADGKNWTDLAATETIAAQESSDRVKPYTYDFAPVGATFVKVTVTNADTTTPSGVVCAGLTEIELKTATSKFVTNTSAALSSLTVNGTKVSDSVLAAGSYNTPAIIADVKAEGEGNASVTVLPAHDNVIRVITESEDHVTRKTFTINLGTEQEFPADSDERDYPAADMTVTVGSEQTSGTATEGPKKFAVDGNTSTYWHSNWTPTTVNDLWIAFELQKPTKLDALRYLPRPAGSKNGSVTEYKVQVSDDGTNWTDAGSGTWTTDYGWKLAEFNQPVTTKHVRLKAVHTYADSGNDKFMSASEIRLRKAVDTTDISGATVTVPAKLTVDRVDADHPATFATKDVTVTLGDATLRYGVDYLLDYAGNTAVGKATVTVRGIDKYSGTVAKTFTIELKNAPAPEPTLTSVSVKTKPSKLTYVVGDAFDPAGLVLQHDRQADRPPQPLVGEQADERGLTCGTRCDRVEQLRKHENREAHRTGLDHLEFVGAADGAVGEQATFKVHVHADQGDGRHDDADERDIDPHVPVDHAVGELARAACHHVIGLRVDTHRLKASGFQIPADDMAEIDRITGFHRFERHVG

SEQ ID NO: 5 - protein, 1935 aa, Artificial sequence
  Artificial sequence
MAVRRLGGRIVAFAATVALSIPLGLLTNSAWAVEDATRSDSTTQMSSTPEVVYSSAVDSKQNRTSDFDANWKFMLSDSVQAQDPAFDDSAWQQVDLPHDYSITQKYSQSNEAESAYLPGGTGWYRKSFTIDRDLAGKRIAINFDGVYMNATVWFNGVKLGTHPYGYSPFSFDLTGNAKFGGENTIVVKVENRLPSSRWYSGSGIYRDVTLTVTDGVHVGNNGVAIKTPSLATQNGGNVTMNLTTKVANDTKAAANITLKQTVFPKGGKTDAAIGTVTTASKSIAAGASADVTSTITAASPKLWSIKNPNLYTVRTEVLNGGKVLDTYDTEYGFRWTGFDATSGFSLNGEKVKLKGVSMHHDQGSLGAVANRRAIERQVEILQKMGVNSIRTTHNPAAKALIDVCNEKGVLVVEEVFDMWNRSKNGNTEDYGKWFGQAIAGDNAVLGGDKDETWAKFDLTSTINRDRNAPSVIMWSLGNEMMEGISGSVSGFPATSAKLVAWTKAADSTRPMTYGDNKIKANWNESNTMGDNLTANGGVVGTNYSDGANYDKIRTTHPSWAIYGSETASAINSRGIYNRTTGGAQSSDKQLTSYDNSAVGWGAVASSAWYDVVQRDFVAGTYVWTGFDYLGEPTPWNGTGSGAVGSWPSPKNSYFGIVDTAGFPKDTYYFYQSQWNDDVHTLHILPAWNENVVAKGSGNNVPVVVYTDAAKVKLYFTPKGSTEKRLIGEKSFTKKTTAAGYTYQVYEGADKDSTAHKNMYLTWNVPWAEGTISAEAYDENNRLIPEGSTEGNASVTTTGKAAKLKADADRKTITADGKDLSYIEVDVTDANGHIVPDAANRVTFDVKGAGKLVGVDNGSSPDHDSYQADNRKAFSGKVLAIVQSTKEAGEITVTAKADGLQSSTVKIATTAVPGTSTEKTVRSFYYSRNYYVKTGNKPILPSDVEVRYSDGTSDRQNVTWDAVSDDQIAKAGSFSVAGTVAGQKISVRVTMIDEIGALLNYSASTPVGTPAVLPGSRPAVLPDGTVTSANFAVDWTKPADTVYNTAGTVKVPGTATVFGKEFKVTATIRVQRSQVTIGSSVSGNALRLTQNIPADKQSDTLDAIKDGSTTVDANTGGGANPSAWTNWAYSKAGHNTAEITFEYATEQQLGQIVMYFFRDSNAVRFPDAGKTKIQISADGKNWTDLAATETIAAQESSDRVKPYTYDFAPVGATFVKVTVTNADTTTPSGVVCAGLTEIELKTATSKFVTNTSAALSSLTVNGTKVSDSVLAAGSYNTPAIIADVKAEGEGNASVTVLPAHDNVIRVITESEDHVTRKTFTINLGTEQEFPADSDERDYPAADMTVTAGSEQTSGTATEGPKKFAVDGNTSTYWHSNWTPTTVNDLWIAFELQKPTKLDALRYLPRPAGSKNGSVTEYKVQVSDDGTNWTDAGSGTWTTDYGWKLAEFNQPVTTKHVRLKAVHTYADSGNDKFMSASEIRLRKAVDTTDISGATVTVPAKLTVDRVDADHPATFATKDVTVTLGDATLRYGVDYLLDYAGNTAVGKATVTVRGIDKYSGTVAKTFTIELKNAPAPEPTLTSVSVKTKPSKLTYVVGDAFDPAGLVLQLNYDDDSTGTVTWNTQTAGDFTFKPALDAKLKVTDKTVTVTYQGKSAVIDITVSQPAPTVSKTDLDKAIKAIEAKNPDSSKYTADSWKTFADAMAHAKAVIADDSATQQDVDKALKALTDAYAGLTEKTPEPAPVSKSELDKKIKAIEAEKLDGSKYTAESWKAFETALAHAKAVIASDSATQQDVDAALGALTSARDGLTEKGEVKPDPKPEPGTVDKAALDKAVKKVEAEKLDGSKYTADSWKAFETALAHAKAVIGNANSTQFDIDNALSMLNDARAALKEKPGRIIAIIDGGALSKTGASVAIIASVAAAMKAVGAGVMALRPPKW

SEQ ID NO: 6 - protein, 887 aa, Bifidobacterium bifidum
VEDATRSDSTTQMSSTPEVVYSSAVDSKQNRTSDFDANWKFMLSDSVQAQDPAFDDSAWQQVDLPHDYSITQKYSQSNEAESAYLPGGTGWYRKSFTIDRDLAGKRIAINFDGVYMNATVWFNGVKLGTHPYGYSPFSFDLTGNAKFGGENTIVVKVENRLPSSRWYSGSGIYRDVTLTVTDGVHVGNNGVAIKTPSLATQNGGDVTMNLTTKVANDTEAAANITLKQTVFPKGGKTDAAIGTVTTASKSIAAGASADVTSTITAASPKLWSIKNPNLYTVRTEVLNGGKVLDTYDTEYGFRWTGFDATSGFSLNGEKVKLKGVSMHHDQGSLGAVANRRAIERQVEILQKMGVNSIRTTHNPAAKALIDVCNEKGVLVVEEVFDMWNRSKNGNTEDYGKWFGQAIAGDNAVLGGDKDETWAKFDLTSTINRDRNAPSVIMWSLGNEMMEGISGSVSGFPATSAKLVAWTKAADSTRPMTYGDNKIKANWNESNTMGDNLTANGGVVGTNYSDGANYDKIRTTHPSWAIYGSETASAINSRGIYNRTTGGAQSSDKQLTSYDNSAVGWGAVASSAWYDVVQRDFVAGTYVWTGFDYLGEPTPWNGTGSGAVGSWPSPKNSYFGIVDTAGFPKDTYYFYQSQWNDDVHTLHILPAWNENVVAKGSGNNVPVVVYTDAAKVKLYFTPKGSTEKRLIGEKSFTKKTTAAGYTYQVYEGSDKDSTAHKNMYLTWNVPWAEGTISAEAYDENNRLIPEGSTEGNASVTTTGKAAKLKADADRKTITADGKDLSYIEVDVTDANGHIVPDAANRVTFDVKGAGKLVGVDNGSSPDHDSYQADNRKAFSGKVLAIVQSTKEAGEITVTAKADGLQSSTVKIATTAVPGTSTEKT

SEQ ID NO: 7 - protein, 965 aa, Bifidobacterium bifidum
VEDATRSDSTTQMSSTPEVVYSSAVDSKQNRTSDFDANWKFMLSDSVQAQDPAFDDSAWQQVDLPHDYSITQKYSQSNEAESAYLPGGTGWYRKSFTIDRDLAGKRIAINFDGVYMNATVWFNGVKLGTHPYGYSPFSFDLTGNAKFGGENTIVVKVENRLPSSRWYSGSGIYRDVTLTVTDGVHVGNNGVAIKTPSLATQNGGDVTMNLTTKVANDTEAAANITLKQTVFPKGGKTDAAIGTVTTASKSIAAGASADVTSTITAASPKLWSIKNPNLYTVRTEVLNGGKVLDTYDTEYGFRWTGFDATSGFSLNGEKVKLKGVSMHHDQGSLGAVANRRAIERQVEILQKMGVNSIRTTHNPAAKALIDVCNEKGVLVVEEVFDMWNRSKNGNTEDYGKWFGQAIAGDNAVLGGDKDETWAKFDLTSTINRDRNAPSVIMWSLGNEMMEGISGSVSGFPATSAKLVAWTKAADSTRPMTYGDNKIKANWNESNTMGDNLTANGGVVGTNYSDGANYDKIRTTHPSWAIYGSETASAINSRGIYNRTTGGAQSSDKQLTSYDNSAVGWGAVASSAWYDVVQRDFVAGTYVWTGFDYLGEPTPWNGTGSGAVGSWPSPKNSYFGIVDTAGFPKDTYYFYQSQWNDDVHTLHILPAWNENVVAKGSGNNVPVVVYTDAAKVKLYFTPKGSTEKRLIGEKSFTKKTTAAGYTYQVYEGSDKDSTAHKNMYLTWNVPWAEGTISAEAYDENNRLIPEGSTEGNASVTTTGKAAKLKADADRKTITADGKDLSYIEVDVTDANGHIVPDAANRVTFDVKGAGKLVGVDNGSSPDHDSYQADNRKAFSGKVLAIVQSTKEAGEITVTAKADGLQSSTVKIATTAVPGTSTEKTVRSFYYSRNYYVKTGNKPILPSDVEVRYSDGTSDRQNVTWDAVSDDQIAKAGSFSVAGTVAGQKISVRVTMIDEIGAL

SEQ ID NO: 8 - protein, 1038 aa, Bifidobacterium bifidum
VEDATRSDSTTQMSSTPEVVYSSAVDSKQNRTSDFDANWKFMLSDSVQAQDPAFDDSAWQQVDLPHDYSITQKYSQSNEAESAYLPGGTGWYRKSFTIDRDLAGKRIAINFDGVYMNATVWFNGVKLGTHPYGYSPFSFDLTGNAKFGGENTIVVKVENRLPSSRWYSGSGIYRDVTLTVTDGVHVGNNGVAIKTPSLATQNGGDVTMNLTTKVANDTEAAANITLKQTVFPKGGKTDAAIGTVTTASKSIAAGASADVTSTITAASPKLWSIKNPNLYTVRTEVLNGGKVLDTYDTEYGFRWTGFDATSGFSLNGEKVKLKGVSMHHDQGSLGAVANRRAIERQVEILQKMGVNSIRTTHNPAAKALIDVCNEKGVLVVEEVFDMWNRSKNGNTEDYGKWFGQAIAGDNAVLGGDKDETWAKFDLTSTINRDRNAPSVIMWSLGNEMMEGISGSVSGFPATSAKLVAWTKAADSTRPMTYGDNKIKANWNESNTMGDNLTANGGVVGTNYSDGANYDKIRTTHPSWAIYGSETASAINSRGIYNRTTGGAQSSDKQLTSYDNSAVGWGAVASSAWYDVVQRDFVAGTYVWTGFDYLGEPTPWNGTGSGAVGSWPSPKNSYFGIVDTAGFPKDTYYFYQSQWNDDVHTLHILPAWNENVVAKGSGNNVPVVVYTDAAKVKLYFTPKGSTEKRLIGEKSFTKKTTAAGYTYQVYEGSDKDSTAHKNMYLTWNVPWAEGTISAEAYDENNRLIPEGSTEGNASVTTTGKAAKLKADADRKTITADGKDLSYIEVDVTDANGHIVPDAANRVTFDVKGAGKLVGVDNGSSPDHDSYQADNRKAFSGKVLAIVQSTKEAGEITVTAKADGLQSSTVKIATTAVPGTSTEKTVRSFYYSRNYYVKTGNKPILPSDVEVRYSDGTSDRQNVTWDAVSDDQIAKAGSFSVAGTVAGQKISVRVTMIDEIGALLNYSASTPVGTPAVLPGSRPAVLPDGTVTSANFAVHWTKPADTVYNTAGTVKVPGTATVFGKEFKVTATIRVQ

SEQ ID NO: 9 - protein, 1142 aa, Bifidobacterium bifidum
VEDATRSDSTTQMSSTPEVVYSSAVDSKQNRTSDFDANWKFMLSDSVQAQDPAFDDSAWQQVDLPHDYSITQKYSQSNEAESAYLPGGTGWYRKSFTIDRDLAGKRIAINFDGVYMNATVWFNGVKLGTHPYGYSPFSFDLTGNAKFGGENTIVVKVENRLPSSRWYSGSGIYRDVTLTVTDGVHVGNNGVAIKTPSLATQNGGDVTMNLTTKVANDTEAAANITLKQTVFPKGGKTDAAIGTVTTASKSIAAGASADVTSTITAASPKLWSIKNPNLYTVRTEVLNGGKVLDTYDTEYGFRWTGFDATSGFSLNGEKVKLKGVSMHHDQGSLGAVANRRAIERQVEILQKMGVNSIRTTHNPAAKALIDVCNEKGVLVVEEVFDMWNRSKNGNTEDYGKWFGQAIAGDNAVLGGDKDETWAKFDLTSTINRDRNAPSVIMWSLGNEMMEGISGSVSGFPATSAKLVAWTKAADSTRPMTYGDNKIKANWNESNTMGDNLTANGGVVGTNYSDGANYDKIRTTHPSWAIYGSETASAINSRGIYNRTTGGAQSSDKQLTSYDNSAVGWGAVASSAWYDVVQRDFVAGTYVWTGFDYLGEPTPWNGTGSGAVGSWPSPKNSYFGIVDTAGFPKDTYYFYQSQWNDDVHTLHILPAWNENVVAKGSGNNVPVVVYTDAAKVKLYFTPKGSTEKRLIGEKSFTKKTTAAGYTYQVYEGSDKDSTAHKNMYLTWNVPWAEGTISAEAYDENNRLIPEGSTEGNASVTTTGKAAKLKADADRKTITADGKDLSYIEVDVTDANGHIVPDAANRVTFDVKGAGKLVGVDNGSSPDHDSYQADNRKAFSGKVLAIVQSTKEAGEITVTAKADGLQSSTVKIATTAVPGTSTEKTVRSFYYSRNYYVKTGNKPILPSDVEVRYSDGTSDRQNVTWDAVSDDQIAKAGSFSVAGTVAGQKISVRVTMIDEIGALLNYSASTPVGTPAVLPGSRPAVLPDGTVTSANFAVHWTKPADTVYNTAGTVKVPGTATVFGKEFKVTATIRVQRSQVTIGSSVSGNALRLTQNIPADKQSDTLDAIKDGSTTVDANTGGGANPSAWTNWAYSKAGHNTAEITFEYATEQQLGQIVMYFFRDSNAVRFPDAGKTKIQI

SEQ ID NO: 10 - protein, 1211 aa, Bifidobacterium bifidum
VEDATRSDSTTQMSSTPEVVYSSAVDSKQNRTSDFDANWKFMLSDSVQAQDPAFDDSAWQQVDLPHDYSITQKYSQSNEAESAYLPGGTGWYRKSFTIDRDLAGKRIAINFDGVYMNATVWFNGVKLGTHPYGYSPFSFDLTGNAKFGGENTIVVKVENRLPSSRWYSGSGIYRDVTLTVTDGVHVGNNGVAIKTPSLATQNGGDVTMNLTTKVANDTEAAANITLKQTVFPKGGKTDAAIGTVTTASKSIAAGASADVTSTITAASPKLWSIKNPNLYTVRTEVLNGGKVLDTYDTEYGFRWTGFDATSGFSLNGEKVKLKGVSMHHDQGSLGAVANRRAIERQVEILQKMGVNSIRTTHNPAAKALIDVCNEKGVLVVEEVFDMWNRSKNGNTEDYGKWFGQAIAGDNAVLGGDKDETWAKFDLTSTINRDRNAPSVIMWSLGNEMMEGISGSVSGFPATSAKLVAWTKAADSTRPMTYGDNKIKANWNESNTMGDNLTANGGVVGTNYSDGANYDKIRTTHPSWAIYGSETASAINSRGIYNRTTGGAQSSDKQLTSYDNSAVGWGAVASSAWYDVVQRDFVAGTYVWTGFDYLGEPTPWNGTGSGAVGSWPSPKNSYFGIVDTAGFPKDTYYFYQSQWNDDVHTLHILPAWNENVVAKGSGNNVPVVVYTDAAKVKLYFTPKGSTEKRLIGEKSFTKKTTAAGYTYQVYEGSDKDSTAHKNMYLTWNVPWAEGTISAEAYDENNRLIPEGSTEGNASVTTTGKAAKLKADADRKTITADGKDLSYIEVDVTDANGHIVPDAANRVTFDVKGAGKLVGVDNGSSPDHDSYQADNRKAFSGKVLAIVQSTKEAGEITVTAKADGLQSSTVKIATTAVPGTSTEKTVRSFYYSRNYYVKTGNKPILPSDVEVRYSDGTSDRQNVTWDAVSDDQIAKAGSFSVAGTVAGQKISVRVTMIDEIGALLNYSASTPVGTPAVLPGSRPAVLPDGTVTSANFAVHWTKPADTVYNTAGTVKVPGTATVFGKEFKVTATIRVQRSQVTIGSSVSGNALRLTQNIPADKQSDTLDAIKDGSTTVDANTGGGANPSAWTNWAYSKAGHNTAEITFEYATEQQLGQIVMYFFRDSNAVRFPDAGKTKIQISADGKNWTDLAATETIAAQESSDRVKPYTYDFAPVGATFVKVTVTNADTTTPSGVVCAGLTEIELKTAT

SEQ ID NO: 11 - protein, 1296 aa, Bifidobacterium bifidum
VEDATRSDSTTQMSSTPEVVYSSAVDSKQNRTSDFDANWKFMLSDSVQAQDPAFDDSAWQQVDLPHDYSITQKYSQSNEAESAYLPGGTGWYRKSFTIDRDLAGKRIAINFDGVYMNATVWFNGVKLGTHPYGYSPFSFDLTGNAKFGGENTIVVKVENRLPSSRWYSGSGIYRDVTLTVTDGVHVGNNGVAIKTPSLATQNGGDVTMNLTTKVANDTEAAANITLKQTVFPKGGKTDAAIGTVTTASKSIAAGASADVTSTITAASPKLWSIKNPNLYTVRTEVLNGGKVLDTYDTEYGFRWTGFDATSGFSLNGEKVKLKGVSMHHDQGSLGAVANRRAIERQVEILQKMGVNSIRTTHNPAAKALIDVCNEKGVLVVEEVFDMWNRSKNGNTEDYGKWFGQAIAGDNAVLGGDKDETWAKFDLTSTINRDRNAPSVIMWSLGNEMMEGISGSVSGFPATSAKLVAWTKAADSTRPMTYGDNKIKANWNESNTMGDNLTANGGVVGTNYSDGANYDKIRTTHPSWAIYGSETASAINSRGIYNRTTGGAQSSDKQLTSYDNSAVGWGAVASSAWYDVVQRDFVAGTYVWTGFDYLGEPTPWNGTGSGAVGSWPSPKNSYFGIVDTAGFPKDTYYFYQSQWNDDVHTLHILPAWNENVVAKGSGNNVPVVVYTDAAKVKLYFTPKGSTEKRLIGEKSFTKKTTAAGYTYQVYEGSDKDSTAHKNMYLTWNVPWAEGTISAEAYDENNRLIPEGSTEGNASVTTTGKAAKLKADADRKTITADGKDLSYIEVDVTDANGHIVPDAANRVTFDVKGAGKLVGVDNGSSPDHDSYQADNRKAFSGKVLAIVQSTKEAGEITVTAKADGLQSSTVKIATTAVPGTSTEKTVRSFYYSRNYYVKTGNKPILPSDVEVRYSDGTSDRQNVTWDAVSDDQIAKAGSFSVAGTVAGQKISVRVTMIDEIGALLNYSASTPVGTPAVLPGSRPAVLPDGTVTSANFAVHWTKPADTVYNTAGTVKVPGTATVFGKEFKVTATIRVQRSQVTIGSSVSGNALRLTQNIPADKQSDTLDAIKDGSTTVDANTGGGANPSAWTNWAYSKAGHNTAEITFEYATEQQLGQIVMYFFRDSNAVRFPDAGKTKIQISADGKNWTDLAATETIAAQESSDRVKPYTYDFAPVGATFVKVTVTNADTTTPSGVVCAGLTEIELKTATSKFVTNTSAALSSLTVNGTKVSDSVLAAGSYNTPAIIADVKAEGEGNASVTVLPAHDNVIRVITESEDHVTRKTFTINLGTEQEF

SEQ ID NO: 12 - protein, 1720 aa, Bifidobacterium bifidum
VEDATRSDSTTQMSSTPEVVYSSAVDSKQNRTSDFDANWKFMLSDSVQAQDPAFDDSAWQQVDLPHDYSITQKYSQSNEAESAYLPGGTGWYRKSFTIDRDLAGKRIAINFDGVYMNATVWFNGVKLGTHPYGYSPFSFDLTGNAKFGGENTIVVKVENRLPSSRWYSGSGIYRDVTLTVTDGVHVGNNGVAIKTPSLATQNGGDVTMNLTTKVANDTEAAANITLKQTVFPKGGKTDAAIGTVTTASKSIAAGASADVTSTITAASPKLWSIKNPNLYTVRTEVLNGGKVLDTYDTEYGFRWTGFDATSGFSLNGEKVKLKGVSMHHDQGSLGAVANRRAIERQVEILQKMGVNSIRTTHNPAAKALIDVCNEKGVLVVEEVFDMWNRSKNGNTEDYGKWFGQAIAGDNAVLGGDKDETWAKFDLTSTINRDRNAPSVIMWSLGNEMMEGISGSVSGFPATSAKLVAWTKAADSTRPMTYGDNKIKANWNESNTMGDNLTANGGVVGTNYSDGANYDKIRTTHPSWAIYGSETASAINSRGIYNRTTGGAQSSDKQLTSYDNSAVGWGAVASSAWYDVVQRDFVAGTYVWTGFDYLGEPTPWNGTGSGAVGSWPSPKNSYFGIVDTAGFPKDTYYFYQSQWNDDVHTLHILPAWNENVVAKGSGNNVPVVVYTDAAKVKLYFTPKGSTEKRLIGEKSFTKKTTAAGYTYQVYEGSDKDSTAHKNMYLTWNVPWAEGTISAEAYDENNRLIPEGSTEGNASVTTTGKAAKLKADADRKTITADGKDLSYIEVDVTDANGHIVPDAANRVTFDVKGAGKLVGVDNGSSPDHDSYQADNRKAFSGKVLAIVQSTKEAGEITVTAKADGLQSSTVKIATTAVPGTSTEKTVRSFYYSRNYYVKTGNKPILPSDVEVRYSDGTSDRQNVTWDAVSDDQIAKAGSFSVAGTVAGQKISVRVTMIDEIGALLNYSASTPVGTPAVLPGSRPAVLPDGTVTSANFAVHWTKPADTVYNTAGTVKVPGTATVFGKEFKVTATIRVQRSQVTIGSSVSGNALRLTQNIPADKQSDTLDAIKDGSTTVDANTGGGANPSAWTNWAYSKAGHNTAEITFEYATEQQLGQIVMYFFRDSNAVRFPDAGKTKIQISADGKNWTDLAATETIAAQESSDRVKPYTYDFAPVGATFVKVTVTNADTTTPSGVVCAGLTEIELKTATSKFVTNTSAALSSLTVNGTKVSDSVLAAGSYNTPAIIADVKAEGEGNASVTVLPAHDNVIRVITESEDHVTRKTFTINLGTEQEFPADSDERDYPAADMTVTVGSEQTSGTATEGPKKFAVDGNTSTYWHSNWTPTTVNDLWIAFELQKPTKLDALRYLPRPAGSKNGSVTEYKVQVSDDGTNWTDAGSGTWTTDYGWKLAEFNQPVTTKHVRLKAVHTYADSGNDKFMSASEIRLRKAVDTTDISGATVTVPAKLTVDRVDADHPATFATKDVTVTLGDATLRYGVDYLLDYAGNTAVGKATVTVRGIDKYSGTVAKTFTIELKNAPAPEPTLTSVSVKTKPSKLTYVVGDAFDPAGLVLQHDRQADRPPQPLVGEQADERGLTCGTRCDRVEQLRKHENREAHRTGLDHLEFVGAADGAVGEQATFKVHVHADQGDGRHDDADERDIDPHVPVDHAVGELARAACHHVIGLRVDTHRLKASGFQIPADDMAEIDRITGFHRFERHVG

SEQ ID NO: 13 - protein, 1396 aa, Bacillus circulans
MRRINFNDNWRFQREISTSLREAQKPSFNDHSWRQLSLPHDWSIELDFNKDSLATHEGGYLDGGVGWYRKTFTVPSAMEGKRISLDFDGVYMNSTTYLNGEELGTYPFGYNAFSYDITDKLFMDGRENVLAVKVDNTQPSSRWYSGSGIYRNVYLTVTNPVHVARYGTFVTTPDLESAYAARKAEVNIKTKINNDSDAAVQVKVKSTIYDTDGKEVASVVSQEKTAAAGTTAHFEDNTVIENPELWSLDNPYRYKLVTDVLIGGETVDTYETRFGARFFKFDANEGFSLNGKPMKLYGVSMHHDLGALGAATNARAVERQLQIMKDMGVNAIRGTHNPVSPEFLEAVNNLGLLLIEEAFDCWSQSKKTYDYGRFFTRWAEHDVKEMVDRGKNEPSIIMWSIGNEIYDTTSPSGVETARNLVRWIKEIDTTRPTTIGEDKTRGDKVNVTPIDPNILEIFHTVDVVGLNYSENNYVGYHEQHPNWKLYGSETSSATRSRGVYTHPYEYNLGTKYDDLQQSSYDNDYVPWGRTAEDAWKSDRDLKHFAGQFIWTGFDYIGEPTPYYDSYPAKSSYFGAVDTAGFPKDIFYYYQSQWKKEPMVHLLPHWNWTEGEPVRVLAYTNAHQVELFLNGKSLGVRGYENKKTSWGAPYKETKDGKTYLEWAVPFKAGTLEAVAMDENGKEIARDQVTTAGAPAAVKLTADRKVIKADGTDLSFITAEIVDSKGNVVPNADHLIQFHLSGHGELAGVDNGDAASVERYKDNKRKAFSGKALAIVQSNKLDGNITLHASAEGLSSGNVTIFTTASADQNSITIAGIDEVNVLVDFNVVPELPSQIKVYYSDSTVEMKPVTWDAVDPNLLNTAGKIIVEGTVEGTDKKAKALLIVKGNGQENSEYRIDLFSPDPKLISTELTVEKTNIMEDDFIDIKVIGQLENKEVVDLSNFMPIYEFDCDIIKIEGNKLYALEEGLVKVTAAVTYKGRTVTSPEMMLKITKNPVPKTITHIDSITVVAGKGEAPVLPATAVAHFDRGMPRDVKVKWEIVNPALYQNLGEFTVSGDVEGTEIKAQAKVMVRSALAIETISMAVLPNQKPELPQKVTVYYSDGTEEQADVDWDAMPSAELKSEGVVKVKGSVKGVDLKATAQIRVTSEVGGVQNISRAKNGYEYPKAEASFTNTGPGSNDRIEAINDDVISYDAEPHNRWTNWQPTPRPGDWVSITFGDSKPRKYDIDSMEIHWYEDLGTSSPAYFRIQYKSGDEWKDVSGLKTNPSNTVLRQANVYTFDKVRTSAIRVDMTAKTGKSLAITEIKVFSKWAKAHTHPMVTDIKLGDLSILDDFSKKGDNNELTFQVKDPRDIPEIKVKAEDNTSITIIPTFTAPSTAKIIAKSEDGMKVEIYNIRFTE

SEQ ID NO: 14 - protein, 1737 aa, Bacillus species
MKKAISCVFLISALILSSFQVPVQGQAMSKTTSAAGNSVSYDGERRVNFNENWRFQRETNGSIAGAQNPGFDDSSWRKLNLPHDWSIELDFNKNSLATHEGGYLDGGIGWYRKTFTIPESMKGKRISLDFDGVYMNSTTYLNGEVLGTYPFGYNAFSYDISDKLYKDGRANVLVVKVNNTQPSSRWYSGSGIYRNVYLTVTDPIHVARYGTFVTTPNLEKSIKEDRADVNIKTKISNDAAEAKQVKIKSTIYDGAGNTVQTVETEEKTAAAGTVTPFEQNTVIKQPKLWSIDKPYRYNLVTEVIVGGQTVDTYETKFGVRYFKFDENEGFSLNGEYMKLHGVSMHHDLGALGAATNARGVERQMQIMKDMGVNAIRVTHNPASPELLEAANKLGLFIIEEAFDSWAQSKKPYDYGRFFNAWAEHDIKEMVDRGKNEPAIIMWSIGNEIYDTTNAAGVETARNLVGWVKEIDTTRPTTIGEDKTRGDKVNVTPINSYIKEIFNIVDVVGLNYSENNYDGYHKQNPSWKLYGSETSSATRSRGVYTHPYQYNQSTKYADLQQSSYDNDYVGWGRTAEDAWKYDRDLKHIAGQFIWTGFDYIGEPTPYYNSYPAKSSYFGAVDTAGFPKDIFYYYQSQWKKEPMVHLLPHWNWKEGEKVRVLAYTNASKVELVLNGESLGEKNYDNKQTSWGAPYKETKDGKTYLEWAVPFKPGKLEAVAKDENGKVIARDQVVTAGEPASVRLTADRKVVKADGTDLSFITADIVDSKGIVVPDADHLITFNVTGQGELAGVDNGNASSVERYKDNKRKAFSGKALAIVQSSKLSGKITVHASVAGLSSDSTSVFTVTPADHDKKIVAGIDDVNLTVDVNEAPKLPSEIKVYYSDESAAAKNVTWDEVDPKQYSTVGEFTVEGSVEGTSLKAKAFVIVKGIVAVKPYSTATKVGVQPVLPEKATLLYSDGTTKGATVTWDEIPEDKLAKEGRFTVEGSVEGTDLKANVYVRVTNEVKSVNIMLQEQGSAYPKLEATFTNPADNLQHLNDGIKSYTNNPVNRWTNWTRTPRDAGDSITVNFGKKHVINNLDLFVFTDSGTVVPEKAEVQYWDGTAWKDVENLTQPSPYVVEKNELTFDAVATEKLKFHLTPSVKGKFLALTEAEVYADQIVMGETAKLQSITVNGKALEGFDHAKKNYELVLPYGSELPKIEAAAADNATVTILPAFSYPGTAKLFVTSEDGKVTTEYSIGVSTEEPKLVSAELSADKTNVMEDDIIDLKVIGLFESKEKIDVTDSQPTYEFDQQIIKIEGNKLYALETGNVKVKVTVTYKGVSVTTPALEFTIAKNPAPKYITSLEPVTVVVKKGEAPELPATVVAHYNRGIPRDVKVKWERINPSKYQQLGEFTVSGMVEGTDIKAQAKVIVKGAVAVEDIRMAVLLKQMPQLPGKVTVYYSDGAEEQRAVKWEEIPQEELENVGEFKVKGDVNGVKLKATATIRVTDEVGGEQNISRAKNGYEYPKAEASFTNNGPGSSDRIEAINDDVISYEANPHNRWTNWQPVPRAGDWVSITFGDYEPTEYDVDSMEIHWFADHGTSYPERFQIEYKSGDSWKEVTSLKSDPASPALGKANVYSFDRVKTSAIRVKMTAQAGKSLAITELKVFSKWPKAGTEPEVTDIKVGGKSILEDFEQKGDHYEVTIDAGDANVMPKINVKAKDQTSITIVPAVTSPSTAKVIAKSEDGKKVKVYSIHYK

SEQ ID NO: 15 - protein, 1025 aa, Kluyveromyces lactis
MSCLIPENLRNPKKVHENRLPTRAYYYDQDIFESLNGPWAFALFDAPLDAPDAKNLDWETAKKWSTISVPSHWELQEDWKYGKPIYTNVQYPIPIDIPNPPTVNPTGVYARTFELDSKSIESFEHRLRFEGVDNCYELYVNGQYVGFNKGSRNGAEFDIQKYVSEGENLVVVKVFKWSDSTYIEDQDQWWLSGIYRDVSLLKLPKKAHIEDVRVTTTFVDSQYQDAELSVKVDVQGSSYDHINFTLYEPEDGSKVYDASSLLNEENGNTTFSTKEFISFSTKKNEETAFKINVKAPEHWTAENPTLYKYQLDLIGSDGSVIQSIKHHVGFRQVELKDGNITVNGKDILFRGVNRHDHHPRFGRAVPLDFVVRDLILMKKFNINAVRNSHYPNHPKVYDLFDKLGFWVIDEADLETHGVQEPFNRHTNLEAEYPDTKNKLYDVNAHYLSDNPEYEVAYLDRASQLVLRDVNHPSIIIWSLGNEACYGRNHKAMYKLIKQLDPTRLVHYEGDLNALSADIFSFMYPTFEIMERWRKNHTDENGKFEKPLILCEYGHAMGNGPGSLKEYQELFYKEKFYQGGFIWEWANHGIEFEDVSTADGKLHKAYAYGGDFKEEVHDGVFIMDGLCNSEHNPTPGLVEYKKVIEPVHIKIAHGSVTITNKHDFITTDHLLFIDKDTGKTIDVPSLKPEESVTIPSDTTYVVAVLKDDAGVLKAGHEIAWGQAELPLKVPDFVTETAEKAAKINDGKRYVSVESSGLHFILDKLLGKIESLKVKGKEISSKFEGSSITFWRPPTNNDEPRDFKNWKKYNIDLMKQNIHGVSVEKGSNGSLAVVTVNSRISPVVFYYGFETVQKYTIFANKINLNTSMKLTGEYQPPDFPRVGYEFWLGDSYESFEWLGRGPGESYPDKKESQRFGLYDSKDVEEFVYDYPQENGNHTDTHFLNIKFEGAGKLSIFQKEKPFNFKISDEYGVDEAAHACDVKRYGRHYLRLDHAIHGVGSEACGPAVLDQYRLKAQDFNFEFDLAFE